European Patent Application EP 4 644 543 A1, published November 5, 2025. Title: SPLINT SEQUENCE AND USE THEREOF IN NUCLEIC ACID CAPTURE. Applicant: BGI SHENZHEN. The sequence listing filed with the application follows.

SEQUENCE LISTING (5 sequences)

SEQ ID NO: 1 - DNA, 22 bp, synthetic construct
  source 1..22: mol_type = other DNA
ttgtcttcctaagaccgcttgg

SEQ ID NO: 2 - DNA, 44 bp, synthetic construct
  source 1..44: mol_type = other DNA
cctccgactgtgtgacttagacttgcacttgatgtgctnnnnnn

SEQ ID NO: 3 - DNA, 45 bp, synthetic construct
  source 1..45: mol_type = other DNA
caagtgcaagtctaagtcacacagtcggaggccaagcggtcttag

SEQ ID NO: 4 - DNA, 44 bp, synthetic construct
  source 1..44: mol_type = other DNA
tctccgactgtgtgactatgacttgaaattaatgtgctnnnnnn

SEQ ID NO: 5 - DNA, 44 bp, synthetic construct
  source 1..44: mol_type = other DNA
aatttcaagtcatagtcacacagtcggagaccaagcggtcttag